European Patent Application EP 4 703 476 A1, published March 4, 2026. Title: PROCESS FOR THE PREPARATION OF OPTICALLY PURE ALKYL DIOLS AND DERIVATIVES THEREOF. Applicant: Technische Universität Graz. Application EP. The sequence listing filed with the application follows.

SEQUENCE LISTING (18 sequences)

SEQ ID NO: 1 - protein, 401 aa, Pseudomonas putida
MLEKHRVLDSAPEYVDKKKYLWILSTLWPATPMIGIWLANETGWGIFYGLVLLVWYGALPLLDAMFGEDFNNPPEEVVPKLEKERYYRVLTYLTVPMHYAALIVSAWWVGTQPMSWLEIGALALSLGIVNGLALNTGHELGHKKETFDRWMAKIVLAVVGYGHFFIEHNKGHHRDVATPMDPATSRMGESIYKFSIREIPGAFIRAWGLEEQRLSRRGQSVWSFDNEILQPMIITVILYAVLLALFGPKMLVFLPIQMAFGWWQLTSANYIEHYGLLRQKMEDGRYEHQKPHHSWNSNHIVSNLVLFHLQRHSDHHAHPTRSYQSLRDFPGLPALPTGYPGAFLMAMIPQWFRSVMDPKVVDWAGGDLNKIQIDDSMRETYLKKFGTSSAGHSSSTSAVAS

SEQ ID NO: 2 - protein, 404 aa, Marinobacter sp.
MSENVLTESLQRDPGAENYVDRKRHLWILSVLWPATPLIGLYLVAQTGWSIWYGLVLILWYGAVPLIDAMFGEDFSNPPESAVPRLEQDRYYRVLTYLTVPIHYAALIVSAWWVSTQPMSVFEFLALALSLGIVNGLALNTGHELGHKKETFDRWMAKLVLAVVGYGHFFIEHNKGHHRDVATPMDPATSRMGESIYSFSLREIPGAFKRAWDLEEQRLSRCGKSVWSLENEVLQPMILTAVLYAGLLAFFGPLMLIFLPIQMAFGWWQLTSANYIEHYGLLREKMSDGRYERQQPHHSWNSNHIMSNLILFHLQRHSDHHAHPTRSYQSLRDFKDLPSLPSGYPGMFLAAMFPSWFRSIMDHRVLDWAKGDLDKIQIQPGKREFYVRKFGGTDSESVDTAASK

SEQ ID NO: 3 - protein, 404 aa, Alcanivorax borkumensis
MSENILTEPPRSDADNEGYVDRKRHLWILSVLWAATPIIGLYLVSQTGWSIWYGLVLILWYGLVPLIDTMLGEDYSNPPESVVPKLEQDRYYKVLTYLTVPIHYAALIISAWWVSTQPIGVFEFLALALSLGIVNGLALNTGHELGHKKETFDRWMAKLVLAVVGYGHFFIEHNKGHHRDVATPMDPATSRMGESIYTFSLREIPGAFKRAWGLEEQRLSRCGKSVWSLDNEVLQPMILTVVLYAALLAFFGPLMLIFLPIQMAFGWWQLTSANYIEHYGLLREKLPNGRYEHQKPHHSWNSNHVMSNLILFHLQRHSDHHAHPTRSYQSLRDFSDLPTLPTGYPGMFFVAFFPSWFRSLMDDRVMEWAHGDINKIQIQPGMREFYEQKFGVKGSESPDTTVAK

SEQ ID NO: 4 - protein, 402 aa, Pseudomonas sp.
MNGKSSVLDSAPEYVDKKKYFWILSTFWPATPMIGIWLANETGWGIFYGLVLAVWYGVLPLLDAMFGEDFNNPPEEVVEKLEKERYYRVLTYLTVPMHYAALIVSAWWVGTQSMSWFEIVALALSLGIVNGLALNTGHELGHKKEAFDRWMAKIVLAVVGYGHFFIEHNKGHHRDVATPMDPATSRMGENIYKFSTREIPGAFRRAWGLEEQRLSRRGQSVWSFDNEILQPMVITVVLYTLLLAFFGPKMLVFLPIQMAFGWWQLTSANYIEHYGLLREKMADGRYEHQKPHHSWNSNHIVSNLVLFHLQRHSDHHAHPTRSYQSLRDFPGLPALPTGYPGAFLMAMIPQWFRSVMDPKVVNWANGDLSKIQIEDSMRAEYIKKFTHNVGADDKRGATAVAS

SEQ ID NO: 5 - protein, 468 aa, Fontimonas thermophila
MSTPTLDAGTLAWNDGKRYLWLLSPFIPVLGLIGLGLFLYTDIGLFTWSGPLLIYGLIPLLDWLVGEDRNNPPEAAVAQLENDRYYRAIVYAYLPTQYAVTVLGTWVAVTADLAIWEYIGLVLSVGAVNGIGINTAHELGHKRENLDRWLAKLTLAPVAYGHFFVEHNRGHHKNVATPEDPASSKMGESFWAFLPRTVIGSLRSAWAIEKARLQRNKQSVWSLDNENLQAWAMTIVLFGALTACLGWPALLFLVLQAAYGASLLEVINYIEHYGLLRQKLPDGRYERCQPRHSWNSNHIVTNLFLYQLQRHSDHHANPTRRFQALRHFDDSPQLPSGYASMLIPAYVPWLWFRLMDPLVARHYGGDLTKANLYPPKRAALLARWHRPRPDARRADTQPTDATATPADAAASPGGRYQCTDCGYIYDEAIGCPREGFPPGTPWSQIPDDWSCPDCAVRDKVDFRKLPAA

SEQ ID NO: 6 - protein, 399 aa, Fontimonas thermophila
MATSMGSHPGFGADSSGTIAYRDRKRPFWTLSVLWPVSPLIGIYLAHTTGVGAFFWLTLAVWYLIIPLLDWVLGDDQSNPPEAVVPALESDRYYRILTYLTVPIHYVVLIGSAWYVSTHYGSMTWYDILGLALSVGIVNGLAINTGHELGHKKTELERWLAKIVLAVVGYGHFFIEHNKGHHKDVATPEDPASAPFGQSIYRFALREIPGAIIRAWNSEKERLGRLGHSPWSLQNEVLQPLLITIPLYVGLIAVLGVKIIPFLLIQIVFGWWQLTSANYIEHYGLLRQKLPDGRYERCQPYHSWNSNHVMSNLILFHLQRHSDHHAHPTRRYQSLRDFPDLPTLPSGYPLMFALSYFPPLWRAVMDRRVLDVCGRDARKINIDPNQREKIIHKFNLLTG

SEQ ID NO: 7 - DNA, 1206 bp, Pseudomonas putida
  source 1..1206: mol_type = genomic DNA
atgcttgagaaacacagagttctggattccgctccagagtacgtagataaaaagaaatatctctggatactatcaactttgtggccggctactccgatgatcggaatctggcttgcaaatgaaactggttgggggattttttatgggctggtattgctcgtatggtacggcgcacttccattgcttgatgcgatgtttggtgaggactttaataatccgcctgaagaagtggtgccgaaactagagaaggagcggtactatcgagttttgacatatctaacagttcctatgcattacgctgcattaattgtgtcagcatggtgggtcggaactcagccaatgtcttggcttgaaattggtgcgcttgccttgtcactgggtatcgtgaacggactagcgctcaatacaggacacgaactcggtcacaagaaggagacttttgatcgttggatggccaaaattgtgttggctgtcgtagggtacggtcacttctttattgagcataataagggtcatcaccgtgatgtcgctacaccgatggatcctgcaacatcccggatgggagaaagcatttataagttttcaatccgtgagatcccaggagcatttattcgtgcttgggggcttgaggaacaacgcctttcgcgccgtggccaaagcgtttggagtttcgataatgaaatcctccaaccaatgatcatcacagttattctttacgccgttctccttgccttgtttggacctaagatgctggtgttcctgccgattcaaatggctttcggttggtggcagctgaccagtgcgaactatattgaacattacggcttgctccgtcaaaaaatggaggacggtcgatatgagcatcaaaagccgcaccattcttggaatagtaatcacatcgtctctaatctagtgctgttccaccttcagcggcactcggatcaccacgcgcatccaacacgttcttatcagtcacttcgggattttcccggcctgccggctcttccgacgggttaccctggtgcatttttgatggcgatgattcctcagtggtttagatcagttatggatcccaaggtagtagattgggctggtggtgaccttaataagatccaaattgatgattcgatgcgagaaacctatttgaaaaaatttggcactagtagtgctggtcatagttcgagtacctctgcggtagcatcgtag

SEQ ID NO: 8 - DNA, 1215 bp, Marinobacter sp.
  source 1..1215: mol_type = genomic DNA
atgtcagaaaatgtactaacggaatccctgcaacgcgaccctggtgcggaaaattatgtggaccgaaaacgccacctgtggatcctgtctgttctgtggccagcaacaccgttgataggcctttatctggtcgcccagaccggatggagcatctggtacggcttggtgttgatcctttggtacggcgcagttccgctcattgatgccatgtttggtgaggattttagcaacccgcctgagtcggcggtgcctcgcttagaacaggatcgttactatcgggtactgacctacctcacggttcctattcactatgccgccttgattgtcagtgcgtggtgggtatcaacgcagccaatgagtgttttcgagtttctggcattggcgctgtccctggggatcgtgaatggcctggctctgaacacaggccatgaactgggccataaaaaagaaacgtttgaccgttggatggcgaaacttgttctcgccgtggtaggctatggtcatttcttcatcgaacacaataaggggcatcaccgcgatgtggccaccccgatggatccggcgacttcccgcatgggcgaaagcatttacagcttctcactgcgtgaaattcccggtgctttcaagcgggcatgggatttagaggaacagcgcctcagtcgttgcggtaaaagtgtctggagcctggaaaatgaagttcttcagccgatgattttaaccgcggtgctttatgcgggattactggcgttttttggcccgttaatgctgatctttttgccgattcaaatggcgtttggctggtggcagctgaccagcgccaactacattgagcattacggactactgcgcgagaagatgagcgatggtcgttatgaacgtcagcaaccgcaccacagctggaactcaaaccatattatgtcgaacctgattctgtttcatttacagcgacatagcgaccatcacgcccatccgacccgctcctatcagtcgcttcgcgacttcaaagacctgccgagcttaccatcgggctatccgggtatgttcctggccgcaatgtttccctcatggtttaggtcgattatggaccaccgcgtgctggattgggctaaaggagatctcgataagattcagatccaacccggcaaacgtgaattctacgtgcgtaaattcggtgggactgattctgaaagcgtcgataccgcagcgtctaaataa

SEQ ID NO: 9 - DNA, 1215 bp, Alcanivorax borkumensis
  source 1..1215: mol_type = genomic DNA
atgagcgagaacattttaaccgagccgccacgaagtgatgcggataatgaaggttatgtggatcgcaaacgccacctgtggattctttctgtgctgtgggcagctacaccaattattggcctatatctggtgtcccagactgggtggagtatctggtacggattagtcctgatcttgtggtacggcctcgtcccgctgatcgacaccatgctgggcgaggattattcgaaccctccggaatcggttgttcctaagcttgaacaagaccgctactacaaagttttaacgtacttaaccgttccgattcattatgcggcgttgattataagtgcgtggtgggtgtctacccaaccaataggggtattcgaatttttagctctcgccctgagcctgggcatcgttaatggactggcactgaacactggccatgaactcggccataaaaaagaaacctttgaccgctggatggccaagctggtactggccgtggtcggctatggtcacttcttcatcgaacacaataaagggcaccatcgtgacgtggcaactccgatggacccggctacatcccgcatgggcgaatctatttatacgttttcactgcgtgaaattccgggtgcctttaaacgggcgtggggcttggaagagcagcgcctcagccgttgcggcaaaagcgtgtggagcctagataatgaagtcttacagcctatgattttgacggtagtgctttatgccgcattgctggcgttttttggtccgttaatgctgatctttttgcccattcagatggcgttcggctggtggcagctgaccagcgccaattatattgaacactacggtctgctgcgtgaaaagctgccgaacggtcgctacgagcatcagaaaccgcatcattcatggaacagcaaccatgtgatgtcgaacctcatcctgtttcacctgcagcgtcatagtgatcaccacgcgcatcctacccgctcgtatcaaagccttagggacttcagcgatcttcccaccctgccgacgggctacccaggtatgttcttcgtcgcattctttccctcctggtttcgttcacttatggatgatagagtgatggagtgggcgcacggagatattaataaaatccagattcagccgggcatgcgtgaattctatgaacaaaaatttggagtaaagggttcggagtcaccggatacgaccgttgccaaataa

SEQ ID NO: 10 - DNA, 1209 bp, Pseudomonas sp.
  source 1..1209: mol_type = genomic DNA
atgaatggcaaaagcagcgttctggatagcgcgcccgaatacgtggacaaaaaaaaatatttttggattctgtcgaccttttggccggctactccgatgatcggaatttggctggccaacgagactggctggggtatcttttatggtttagtcctagcagtgtggtatggggtacttccgctgcttgacgcgatgttcggtgaggactttaacaatccgccggaggaagtagtggagaaactggagaaagaacgttactatcgagttttaacgtatcttaccgttccaatgcattacgcagcactgatcgtgtctgcctggtgggtagggacacagtcaatgtcctggttcgaaatcgtcgccctggccttgagtctgggcatcgtgaatggcctagcgctgaacaccggccacgaactgggtcataaaaaagaagcctttgatcgttggatggcgaaaattgtgctggcggttgtcgggtatggccatttctttattgagcataacaaaggccatcaccgtgatgttgcgaccccgatggaccctgcgacctcccgcatgggagaaaatatatataaattctcaacccgcgaaattcctggagcgtttcgtcgtgcttggggcttggaagaacagcgcttatcgcgccgcggccaaagcgtttggagtttcgataatgagatcctccagccaatggtcattacagtggtgctctacaccctcctgcttgccttctttggtccgaagatgctggtgttccttccaattcagatggccttcgggtggtggcagttaacgagcgcgaactacattgaacactacggtttgctgcgtgaaaaaatggccgatggaaggtatgaacatcaaaagcctcatcactcgtggaacagtaaccacatcgtgtctaacctggtcctgtttcacttacagcgccattctgatcaccatgcgcacccgacgcgctcctaccagagcttacgtgatttccccggcctgccggcactcccgactggctaccccggtgcctttttgatggcaatgattccgcaatggtttagatcggtgatggaccctaaggtggtaaattgggctaatggcgacctgagcaagattcagattgaagattcaatgcgcgccgaatatattaaaaagtttacgcataatgttggtgcggatgataaacggggcgcaaccgcggtagcaagctaa

SEQ ID NO: 11 - DNA, 1407 bp, Fontimonas thermophila
  source 1..1407: mol_type = genomic DNA
atgtctacgccgacactggatgcaggaaccttagcttggaacgacgggaaacgttatttgtggttactttccccattcattccggtactgggtctgatcggtcttggtttatttctttataccgatataggtttatttacctggtctggacctctgctgatttatggtttaataccgctgttggattggctggttggcgaggatcgcaataacccaccagaagcggccgttgcgcagttggaaaacgatagatactaccgtgctattgtgtatgcgtacctgccgacccagtatgcggtgacggttctgggcacctgggttgccgtgactgcggacctggcgatttgggagtacattggcctagtcctgtcagtaggcgccgttaacggcattggcattaatactgcacacgaactgggacataaacgtgagaatctggaccgctggctcgcaaagctgaccctcgcaccagtggcgtacggtcacttttttgtggaacacaaccggggacatcataaaaacgttgcgacaccggaggatccggcctcaagcaaaatgggtgaatccttctgggcgttcctgccccgaacggtcattggctcattgcgtagcgcttgggccatcgaaaaagctcgcctgcagcgcaataagcagagcgtgtggtcgctcgataacgaaaatctgcaggcgtgggccatgactatcgtcttatttggcgccctgaccgcatgtctcgggtggccagcgctgctgtttctggtactacaggcagcgtatggcgccagtttacttgaggtgatcaactatattgaacattatggcttgctgcgtcaaaaattgccggacggtcgctatgaacgttgccagccgcgccacagctggaatagcaatcacattgtcaccaacctgtttctctaccagctgcaacgtcattccgatcatcatgcaaacccgactcgcagattccaagccctgcgacatttcgatgacagtcctcaattgccctcgggttacgcctcgatgttaatcccagcgtatgtgccgtggctgtggtttcggctgatggacccgttggtcgctcgtcattatgggggtgacctgaccaaagcaaatctttatccacctaaacgcgcagcacttctggcccgctggcaccgccctcgccccgatgcgcgtcgcgcggatacgcagccgaccgatgctacggcaacaccggccgatgcggctgctagtcccggcggccgttaccaatgcacagactgcggttacatctatgatgaagcgatcggctgtccgcgggaagggttcccgccggggacgccttggtctcagatcccggacgattggagctgccctgattgtgccgtgcgtgacaaggtagattttaggaaactcccggcggcctaa

SEQ ID NO: 12 - DNA, 1200 bp, Fontimonas thermophila
  source 1..1200: mol_type = genomic DNA
atggccacttcaatgggctcccatcctggtttcggtgcagacagctcgggaacaattgcgtatagggatcgtaaacgcccgttctggaccctcagcgttctttggcccgtaagtccgctgatcggaatttaccttgcgcataccactggcgtgggtgccttcttttggctcacgctggcggtttggtacttgattattccgctcctggactgggttcttggtgatgatcaaagcaacccacctgaagcggtggtgccggctttggagtcggatcgctattaccgtattcttacctatttaacggtgccgatacactatgtggtgctaatcggcagtgcgtggtatgtctcgacccactacgggtctatgacgtggtatgatatactcggtctggctctgagtgttggcattgtcaatggtcttgcaattaacacaggccacgaactgggccataaaaaaaccgaactggaacgttggctggcgaagattgtgttggccgtagtggggtacggtcacttttttattgaacataataaaggccatcataaagatgttgctaccccagaagatcccgccagtgcaccatttggtcagtcaatttaccgttttgccctgcgtgaaatccctggcgcgatcatccgtgcctggaacagcgaaaaggagcgcttaggccggctgggtcatagcccgtggtctttacaaaatgaagtgttacaacctctgctgatcacgataccgctatatgttggcctgattgcggtactgggggttaaaattatcccgtttcttctgatccagattgtattcggttggtggcaactgacgtccgccaattatatcgagcattacgggctgctgcgccagaagctgccggatggacgctacgaacgttgtcagccgtatcactcatggaacagcaaccacgtcatgtccaacctgatcttgttccacttacagcgccattccgatcatcatgcacatccgacccgccgttatcagtctttacgagactttccggacctgccgacactcccctcggggtacccattaatgttcgcgctgagctattttcctccgctgtggcgcgctgtcatggacagacgcgtgttggatgtctgcggccgggatgcacggaaaattaatattgacccaaaccagcgagagaaaatcatccacaaatttaatctgttgactggctaa

SEQ ID NO: 13 - protein, 173 aa, Pseudomonas aeruginosa
MASYKCPDCNYVYDESAGNVHEGFSPGTPWHLIPEDWCCPDCAVRDKLDFMLIESGVGEKGVTSTHTSPNLSEVSGTSLTAEAVVAPTSLEKLPSADVKGQDLYKTQPPRSDAQGGKAYLKWICITCGHIYDEALGDEAEGFTPGTRFEDIPDDWCCPDCGATKEDYVLYEEK

SEQ ID NO: 14 - protein, 132 aa, Stutzerimonas degradans
MSRYQCPDCQYIYDENKGEPHEGFHPNTSWNDIPKDWACPDCAVRDKVDFIFLADSPSKETQLGVNSQLANSESGISDATPTGMAVLAAELVIPLNQENKNEGCAAKTEVLDQASTPQVVRKSSTRKKMRNK

SEQ ID NO: 15 - DNA, 522 bp, Pseudomonas aeruginosa
  source 1..522: mol_type = genomic DNA
atggctagctataaatgcccggattgtaattatgtttatgatgagagtgcgggtaatgtgcatgaggggttttctccaggtacgccttggcaccttattcctgaggattggtgctgccccgattgcgccgttcgagacaagcttgacttcatgttaattgagagcggcgtaggtgaaaagggcgtcacctcaacccatacttcgccaaatttatccgaggttagtggcacaagtttaactgctgaagcagtggttgcgccgacaagcttagagaaattgcctagtgccgacgttaaaggccaagatctatataaaactcaacctccaaggtctgatgcccaaggcgggaaagcatacttgaagtggatatgtattacttgtggccatatatatgatgaggcgttgggcgatgaggccgagggttttactccaggtactcgctttgaggatattcctgatgactggtgctgtccggattgcggggctacgaaagaagactatgtgctctacgaggaaaagtga

SEQ ID NO: 16 - DNA, 399 bp, Stutzerimonas degradans
  source 1..399: mol_type = genomic DNA
atgtcaaggtaccagtgtccagattgtcagtatatctatgatgaaaataagggggagccgcacgaaggtttccacccgaacaccagctggaatgatatccccaaagattgggcatgcccggactgcgcagttcgagacaaggtggactttatctttctcgcggattctccctcgaaagaaacacagctaggggtgaatagtcagcttgccaactcggaaagtggtatttcagatgctactccaactggaatggcagttttggccgcagaattagtgatcccacttaatcaagaaaataaaaatgagggctgtgcggctaagactgaagttcttgatcaggcgagcaccccacaggttgtaagaaaatcttccacaaggaagaagatgagaaataaataa

SEQ ID NO: 17 - protein, 385 aa, Pseudomonas oleovorans
MAIVVVGAGTAGVNAAFWLRQYGYKGEIRIFSRESVAPYQRPPLSKAFLTSEIAESAVPLKPEGFYTNNNITISLNTPIVSIDVGRKIVSSKDGKEYAYEKLILATPASARRLTCEGSELSGVCYLRSMEDAKNLRRKLVESASVVVLGGGVIGLEVASAAVGLGKRVTVIEATPRVMARVVTPAAANLVRARLEAEGIEFKLNAKLTSIKGRNGHVEQCVLESGEEIQADLIVVGIGAIPELELATEAALEVSNGVVVDDQMCTSDTSIYAIGDCAMARNPFWGTMVRLETIHNAVTHAQIVASSICGTSTPAPTPPRFWSDLKGMALQGLGALKDYDKLVVAINNETLELEVLAYKQERLIATETINLPKRQGALAGSIKLPD

SEQ ID NO: 18 - DNA, 1158 bp, Pseudomonas oleovorans
  source 1..1158: mol_type = genomic DNA
atggcaatcgttgttgttggcgctggtacagctggagtaaatgctgcgttctggcttcgtcaatatggttataaaggggaaattaggatttttagcagggagtctgtggcgccttatcagcggcctcctctatccaaggcttttctgacaagtgagattgcagaatccgcagtgccattaaagccagaaggtttttatacgaataacaatattaccatttcgttaaatacaccgattgtatcaatcgacgtggggcgtaagatagtttcttctaaagatggaaaagaatacgcgtatgaaaaattgattcttgcaacacctgctagcgcacgtaggttaacctgcgaggggtctgaactgtctggggtctgctatttacgcagtatggaagacgccaaaaatttacgtaggaaacttgtggagagtgcgtctgttgttgtgttgggcggcggagtaatcgggcttgaagtcgcctcagctgcggtgggcttagggaagagggtcacagtgatagaagccaccccgcgtgtaatggcgcgcgtggttacgccggcagcagcaaacttagtcagagcccgcctggaggctgaaggaattgagttcaagctgaatgcgaaattaacgtctataaagggcaggaatggccatgttgaacaatgcgtacttgaaagtggagaagaaattcaggcggatctgattgtagttggaatcggtgctatcccagagctagagctggcaactgaggcggcccttgaagtgagtaatggtgttgtggtcgatgatcagatgtgtacatcggatacaagtatatatgcaatcggcgactgcgcaatggctagaaatcctttttggggaacgatggtacgtttagagacaattcataatgcggttacacacgctcaaattgtcgcaagtagcatctgtggcacatcaacaccagcaccaaccccaccacggttctggtctgatcttaaagggatggcgctgcaaggacttggtgctctaaaggactacgataaactcgttgttgcaattaataacgaaactcttgaactagaagtccttgcgtacaagcaggagcgactgattgcaactgagacaataaatttgcctaaacgtcaaggtgcgcttgcagggagtataaaattacctgattag